European Patent Specification EP 3 810 151 B1, published August 6, 2025. Title: RIG-I Agonists and Treatments Using Same. Applicant: Yale University Iwasaki, Akiko Pyle, Anna Marie Jiang, Xiaodong Fedorova, Olga. The sequence listing filed with the application follows.

SEQUENCE LISTING (17 sequences)

SEQ ID NO: 1 - RNA, 32 nt, Artificial Sequence
  Chemically synthesized
  misc_feature (1)..(1): 5-triphosphorylated
ggaucgaucgaucguucgcgaucgaucgaucc

SEQ ID NO: 2 - RNA, 20 nt, Artificial Sequence
  Chemically synthesized
  misc_feature (1)..(1): 5'-triphosphorylated
ggcgcggcuucggccgcgcc

SEQ ID NO: 3 - RNA, 20 nt, Artificial Sequence
  Chemically synthesized
  misc_feature (1)..(1): 5'-triphosphorylated
ggcgcggguucgcccgcgcc

SEQ ID NO: 4 - RNA, 22 nt, Artificial Sequence
  Chemically synthesized
  misc_feature (1)..(1): 5'-triphosphorylated
ggcgccggguucgcccggcgcc

SEQ ID NO: 5 - RNA, 24 nt, Artificial Sequence
  Chemically synthesized
  misc_feature (1)..(1): 5-triphosphorylated
ggacguacguuucgacguacgucc

SEQ ID NO: 6 - RNA, 20 nt, Artificial Sequence
  Chemically synthesized
  misc_feature (1)..(1): 5'-triphosphorylated
ggcgacguuucgacgucgcc

SEQ ID NO: 7 - RNA, 22 nt, Artificial Sequence
  Chemically synthesized
  misc_feature (1)..(1): 5'-triphosphorylated
ggcguacguuucgacguacgcc

SEQ ID NO: 8 - RNA, 32 nt, Artificial Sequence
  Chemically synthesized
  misc_feature (1)..(1): 5'-triphosphorylated
ggaucgaucgaucggaaccgaucgaucgaucc

SEQ ID NO: 9 - RNA, 32 nt, Artificial Sequence
  Chemically synthesized
  misc_feature (1)..(1): 5'-triphosphorylated
ggaucgaucgaucgcuugcgaucgaucgaucc

SEQ ID NO: 10 - RNA, 33 nt, Artificial Sequence
  Chemically synthesized
  misc_feature (1)..(1): 5'-triphosphorylated
ggaucgaucgaucguuuuucgaucgaucgaucc

SEQ ID NO: 11 - RNA, 35 nt, Artificial Sequence
  Chemically synthesized
  misc_feature (1)..(1): 5'-triphosphorylated
ggaucgaucgaucgacaaugccgaucgaucgaucc

SEQ ID NO: 12 - RNA, 33 nt, Artificial Sequence
  Chemically synthesized
  misc_feature (1)..(1): 5'-triphosphorylated
  misc_feature (15)..(15): abasic ribonucleotide
  misc_feature (16)..(16): abasic ribonucleotide
  misc_feature (17)..(17): abasic ribonucleotide
  misc_feature (18)..(18): abasic ribonucleotide
  misc_feature (19)..(19): abasic ribonucleotide
ggaucgaucgaucgnnnnncgaucgaucgaucc

SEQ ID NO: 13 - RNA, 15 nt, Artificial Sequence
  Chemically synthesized
  misc_feature (1)..(1): 5'-triphosphorylated
ggaucgaucgaucgu

SEQ ID NO: 14 - RNA, 15 nt, Artificial Sequence
  Chemically synthesized
  misc (1)..(1): 5'-triphosphorylated
gcgaucgaucgaucc

SEQ ID NO: 15 - RNA, 12 nt, Artificial Sequence
  Chmeically synthesized
gcccagaccacc

SEQ ID NO: 16 - RNA, 17 nt, Artificial Sequence
  Chemically synthesized
aaaaagguggucugggc

SEQ ID NO: 17 - RNA, 24 nt, Artificial Sequence
  Chemically synthesized
ggacguacguuucgacguacgugg